European Patent Specification EP 3 732 958 B1, published April 19, 2023. Title: Cry1D for Controlling Corn Earworm. Applicant: Agrigenetics, Inc. The sequence listing filed with the application follows.

SEQUENCE LISTING (15 sequences)

SEQ ID NO: 1 - DNA, 3420 bp, artificial
  DIG-911 DNA; Cry1Da2/Cry1Ab chimeric toxin, from pDOW2848
atggaaataaataatcaaaaccaatgtgtgccttacaattgtttaagtaatcctaaggagataatattaggcgaggaaaggctagaaacagggaatactgtagcagacatttcattagggcttattaattttctatattctaattttgtaccaggaggaggatttatagtaggtttactagaattaatatggggatttatagggccttcgcaatgggatatttttttagctcaaattgagcaattgattagtcaaagaatagaagaatttgctaggaatcaggcaatttcaagattggaggggctaagcaatctttataaggtctatgttagagcgtttagcgactgggagaaagatcctactaatcctgctttaagggaagaaatgcgtatacaatttaatgacatgaatagtgctctcataacggctattccactttttagagttcaaaattatgaagttgctcttttatctgtatatgttcaagccgcaaacttacatttatctattttaagggatgtttcagttttcggagaaagatggggatatgatacagcgactatcaataatcgctatagtgatctgactagccttattcatgtttatactaaccattgtgtggatacgtataatcagggattaaggcgtttggaaggtcgttttcttagcgattggattgtatataatcgtttccggagacaattgacaatttcagtattagatattgttgcgttttttccaaattatgatattagaacatatccaattcaaacagctactcagctaacgagggaagtctatctggatttaccttttattaatgaaaatctttctcctgcagcaagctatccaaccttttcagctgctgaaagtgctataattagaagtcctcatttagtagactttttaaatagctttaccatttatacagatagtctggcacgttatgcatattggggagggcacttggtaaattctttccgcacaggaaccactactaatttgataagatcccctttatatggaagggaaggaaatacagagcgccccgtaactattaccgcatcacctagcgtaccaatatttagaacactttcatatattacaggccttgacaattcaaatcctgtagctggaatcgagggagtggaattccaaaatactataagtagaagtatctatcgtaaaagcggtccaatagattcttttagtgaattaccacctcaagatgccagcgtatctcctgcaattgggtatagtcaccgtttatgccatgcaacatttttagaacggattagtggaccaagaatagcaggcaccgtattttcttggacacaccgtagtgccagccctactaatgaagtaagtccatctagaattacacaaattccatgggtaaaggcgcatactcttgcatctggtgcctccgtcattaaaggtcctggatttacaggtggagatattctgactaggaatagtatgggcgagctggggaccttacgagtaaccttcacaggaagattaccacaaagttattatatacgtttccgttatgcttcggtagcaaataggagtggtacatttagatattcacagccaccttcgtatggaatttcatttccaaaaactatggacgcaggtgaaccactaacatctcgttcgttcgctcatacaacactcttcactccaataaccttttcacgagctcaagaagaatttgatctatacatccaatcgggtgtttatatagatcgaattgaatttataccggttactgcaacactggaggcagagtctgacttggaaagagcacagaaggcggtgaatgctctgttcacttcgtccaatcagattgggctcaagacagatgtgactgactatcacatcgatcgcgtttccaaccttgttgagtgcctctctgatgagttctgtttggatgagaagaaggagttgtccgagaaggtcaaacatgctaagcgacttagtgatgagcggaacttgcttcaagatcccaactttcgcgggatcaacaggcaactagatcgtggatggaggggaagtacggacatcaccattcaaggaggtgatgatgtgttcaaggagaactatgttacgctcttgggtacctttgatgagtgctatccaacatacctgtaccagaagatagatgaatcgaaactcaaagcctacacaagataccagttgagaggttacatcgaggacagtcaagaccttgagatctacctcatcagatacaacgccaaacatgagacagtcaatgtgcctgggacgggttcactctggccactttcagccccaagtcccatcggcaagtgtgcccatcactcacaccacttctccttggacatagacgttggctgtaccgacctgaacgaagacctcggtgtgtgggtgatcttcaagatcaagactcaagatggccatgccaggctaggcaatctggagtttctagaagagaaaccacttgttggagaagccctcgctagagtgaagagggctgagaagaagtggagggacaagagagagaagttggaatgggaaacaaacattgtgtacaaagaagccaaagaaagcgttgacgctctgtttgtgaactctcagtatgataggctccaagctgataccaacatagctatgattcatgctgcagacaaacgcgttcatagcattcgggaagcttaccttcctgaacttagcgtgattccgggtgtcaatgctgctatctttgaagagttagaagggcgcatcttcactgcattctccttgtatgatgcgaggaatgtcatcaagaatggtgacttcaacaatggcctatcctgctggaatgtgaaagggcacgtagatgtagaagaacagaacaatcaccgctctgtccttgttgttcctgagtgggaagcagaagtttcacaagaagttcgtgtctgtcctggtcgtggctacattcttcgtgttaccgcgtacaaagaaggatacggagaaggttgcgtcaccatacacgagattgagaacaacaccgacgagctgaagttcagcaactgcgtcgaggaggaagtctacccaaacaacaccgtaacttgcaatgactacactgcgactcaagaggagtatgagggtacttacacttctcgcaatcgaggatacgatggagcctatgagagcaactcttctgtacccgctgactatgcatcagcctatgaggagaaggcttacaccgatggacgtagggacaatccttgcgaatctaacagaggctatggggactacacaccgttaccagccggctatgtcaccaaagagttagagtactttccagaaaccgacaaggtttggattgagattggagaaacggaaggaacattcattgttgatagcgtggagttacttctgatggaggaatga

SEQ ID NO: 2 - protein, 1139 aa, artificial
  amino acid sequence for the DIG-911 protein (Cry1Da2/Cry1Ab chimeric insecticidal toxin, which consists of a core toxin segment of Cry1Da (amino acids 1 to 594, as disclosed in GENBANK Accession No. 176415.1 and U.S Patent No. 5,691,308) and a
MEINNQNQCVPYNCLSNPKEIILGEERLETGNTVADISLGLINFLYSNFVPGGGFIVGLLELIWGFIGPSQWDIFLAQIEQLISQRIEEFARNQAISRLEGLSNLYKVYVRAFSDWEKDPTNPALREEMRIQFNDMNSALITAIPLFRVQNYEVALLSVYVQAANLHLSILRDVSVFGERWGYDTATINNRYSDLTSLIHVYTNHCVDTYNQGLRRLEGRFLSDWIVYNRFRRQLTISVLDIVAFFPNYDIRTYPIQTATQLTREVYLDLPFINENLSPAASYPTFSAAESAIIRSPHLVDFLNSFTIYTDSLARYAYWGGHLVNSFRTGTTTNLIRSPLYGREGNTERPVTITASPSVPIFRTLSYITGLDNSNPVAGIEGVEFQNTISRSIYRKSGPIDSFSELPPQDASVSPAIGYSHRLCHATFLERISGPRIAGTVFSWTHRSASPTNEVSPSRITQIPWVKAHTLASGASVIKGPGFTGGDILTRNSMGELGTLRVTFTGRLPQSYYIRFRYASVANRSGTFRYSQPPSYGISFPKTMDAGEPLTSRSFAHTTLFTPITFSRAQEEFDLYIQSGVYIDRIEFIPVTATLEAESDLERAQKAVNALFTSSNQIGLKTDVTDYHIDRVSNLVECLSDEFCLDEKKELSEKVKHAKRLSDERNLLQDPNFRGINRQLDRGWRGSTDITIQGGDDVFKENYVTLLGTFDECYPTYLYQKIDESKLKAYTRYQLRGYIEDSQDLEIYLIRYNAKHETVNVPGTGSLWPLSAPSPIGKCAHHSHHFSLDIDVGCTDLNEDLGVWVIFKIKTQDGHARLGNLEFLEEKPLVGEALARVKRAEKKWRDKREKLEWETNIVYKEAKESVDALFVNSQYDRLQADTNIAMIHAADKRVHSIREAYLPELSVIPGVNAAIFEELEGRIFTAFSLYDARNVIKNGDFNNGLSCWNVKGHVDVEEQNNHRSVLVVPEWEAEVSQEVRVCPGRGYILRVTAYKEGYGEGCVTIHEIENNTDELKFSNCVEEEVYPNNTVTCNDYTATQEEYEGTYTSRNRGYDGAYESNSSVPADYASAYEEKAYTDGRRDNPCESNRGYGDYTPLPAGYVTKELEYFPETDKVWIEIGETEGTFIVDSVELLLMEE

SEQ ID NO: 3 - DNA, 3447 bp, artificial
  DIG-180 DNA; Cry1Fa2
atggaaaataatattcaaaatcaatgcgtaccttacaattgtttaaataatcctgaagtagaaatactgaacgaagaacgcagcaccggccgcctgccgctggacatcagcctgagccttacacgtttccttttgagtgaatttgttccaggtgtgggagttgcgtttggattatttgatttaatatggggttttataactccttctgattggagcttatttcttttacagattgaacaattgattgagcaaagaatagaaacattggaaaggaaccgggcaattactacattacgagggttagcagatagctatgaaatttatattgaagcactaagagagtgggaagcaaatcctaataatgcacaattaagggaagatgtgcgtattcgatttgctaatacagacgacgctttaataacagcaataaataattttacacttacaagttttgaaatccctcttttatcggtctatgttcaagcggcgaatttacatttatcactattaagagacgcagtatcgtttgggcagggttggggactggatatagctactgttaataatcattataatagattaataaatcttattcatagatatacgaaacattgtttggacacatacaatcaaggattagaaaacttaagaggtactaatactcgacaatgggcaagattcaatcagtttaggagagatttaacacttactgtattagatatcgttgctctttttccgaactacgatgttagaacatatccaattcaaacgtcatcccaattaacaagggaaatttatacaagttcagtaattgaggattctccagtttctgctaatatacctaatggttttaatagggcggaatttggagttagaccgccccatcttatggactttatgaattctttgtttgtaactgcagagactgttagaagtcaaactgtgtggggaggacacttagttagttcacgaaatacggctggtaaccgtataaatttccctagttacggggtcttcaatcctggtggcgccatttggattgcagatgaggatccacgtcctttttatcggacattatcagatcctgtttttgtccgaggaggatttgggaatcctcattatgtactggggcttaggggagtagcatttcaacaaactggtacgaaccacacccgaacatttagaaatagtgggaccatagattctctagatgaaatcccacctcaggataatagtggggcaccttggaatgattatagtcatgtattaaatcatgttacatttgtacgatggccaggtgagatttcaggaagtgattcatggagagctccaatgttttcttggacgcaccgtagtgcaacccctacaaatacaattgatccggagaggattactcaaataccattggtaaaagcacatacacttcagtcaggtactactgttgtaagagggcccgggtttacgggaggagatattcttcgacgaacaagtggaggaccatttgcttatactattgttaatataaatgggcaattaccccaaaggtatcgtgcaagaatacgctatgcctctactacaaatctaagaatttacgtaacggttgcaggtgaacggatttttgctggtcaatttaacaaaacaatggataccggtgacccattaacattccaatcttttagttacgcaactattaatacagcttttacattcccaatgagccagagtagtttcacagtaggtgctgatacttttagttcagggaatgaagtttatatagacagatttgaattgattccagttactgcaacattggaagcagaatctgatttagaaagagcacaaaaggcggtgaatgcgctgtttacttctagcaaccaaatagggctaaaaacagatgtgacggattatcatatcgatcgagtatccaatttagttgagtgtttatctgatgaattttgtctggatgaaaaaaaagaattgtccgagaaagtcaaacatgcgaagcgacttagtgatgagcggaatttacttcaagatccaaactttagagggatcaatagacaactagaccgtggctggagaggaagtacggatattaccatccaaggaggcgatgacgtattcaaagagaattacgttacgctattgggtacctttgatgagtgctatccaacgtatttatatcaaaaaatagatgagtcgaaattaaaagcctatacccgttaccaattaagagggtatatcgaagatagtcaagacttagaaatctatttaattcgctacaatgccaaacacgaaacagtaaatgtgccaggtacgggttccttatggccgctttcagccccaagtccaatcggaaaatgtgcccatcattcccatcatttctccttggacattgatgttggatgtacagacttaaatgaggacttaggtgtatgggtgatattcaagattaagacgcaagatggccatgcaagactaggaaatctagaatttctcgaagagaaaccattagtaggagaagcactagctcgtgtgaaaagagcggagaaaaaatggagagacaaacgtgaaaaattggaatgggaaacaaatattgtttataaagaggcaaaagaatctgtagatgctttatttgtaaactctcaatatgatagattacaagcggataccaacatcgcgatgattcatgcggcagataaacgcgttcatagcattcgagaagcttatctgcctgagctgtctgtgattccgggtgtcaatgcggctatttttgaagaattagaagggcgtattttcactgcattctccctatatgatgcgagaaatgtcattaaaaatggtgattttaataatggcttatcctgctggaacgtgaaagggcatgtagatgtagaagaacaaaacaaccaccgttcggtccttgttgttccggaatgggaagcagaagtgtcacaagaagttcgtgtctgtccgggtcgtggctatatccttcgtgtcacagcgtacaaggagggatatggagaaggttgcgtaaccattcatgagatcgagaacaatacagacgaactgaagtttagcaactgtgtagaagaggaagtatatccaaacaacacggtaacgtgtaatgattatactgcgactcaagaagaatatgagggtacgtacacttctcgtaatcgaggatatgacggagcctatgaaagcaattcttctgtaccagctgattatgcatcagcctatgaagaaaaagcatatacagatggacgaagagacaatccttgtgaatctaacagaggatatggggattacacaccactaccagctggctatgtgacaaaagaattagagtacttcccagaaaccgataaggtatggattgagatcggagaaacggaaggaacattcatcgtggacagcgtggaattacttcttatggaggaataa

SEQ ID NO: 4 - protein, 1148 aa, artificial
  DIG-180 protein; Cry1Fa2
MENNIQNQCVPYNCLNNPEVEILNEERSTGRLPLDISLSLTRFLLSEFVPGVGVAFGLFDLIWGFITPSDWSLFLLQIEQLIEQRIETLERNRAITTLRGLADSYEIYIEALREWEANPNNAQLREDVRIRFANTDDALITAINNFTLTSFEIPLLSVYVQAANLHLSLLRDAVSFGQGWGLDIATVNNHYNRLINLIHRYTKHCLDTYNQGLENLRGTNTRQWARFNQFRRDLTLTVLDIVALFPNYDVRTYPIQTSSQLTREIYTSSVIEDSPVSANIPNGFNRAEFGVRPPHLMDFMNSLFVTAETVRSQTVWGGHLVSSRNTAGNRINFPSYGVFNPGGAIWIADEDPRPFYRTLSDPVFVRGGFGNPHYVLGLRGVAFQQTGTNHTRTFRNSGTIDSLDEIPPQDNSGAPWNDYSHVLNHVTFVRWPGEISGSDSWRAPMFSWTHRSATPTNTIDPERITQIPLVKAHTLQSGTTVVRGPGFTGGDILRRTSGGPFAYTIVNINGQLPQRYRARIRYASTTNLRIYVTVAGERIFAGQFNKTMDTGDPLTFQSFSYATINTAFTFPMSQSSFTVGADTFSSGNEVYIDRFELIPVTATLEAESDLERAQKAVNALFTSSNQIGLKTDVTDYHIDRVSNLVECLSDEFCLDEKKELSEKVKHAKRLSDERNLLQDPNFRGINRQLDRGWRGSTDITIQGGDDVFKENYVTLLGTFDECYPTYLYQKIDESKLKAYTRYQLRGYIEDSQDLEIYLIRYNAKHETVNVPGTGSLWPLSAPSPIGKCAHHSHHFSLDIDVGCTDLNEDLGVWVIFKIKTQDGHARLGNLEFLEEKPLVGEALARVKRAEKKWRDKREKLEWETNIVYKEAKESVDALFVNSQYDRLQADTNIAMIHAADKRVHSIREAYLPELSVIPGVNAAIFEELEGRIFTAFSLYDARNVIKNGDFNNGLSCWNVKGHVDVEEQNNHRSVLVVPEWEAEVSQEVRVCPGRGYILRVTAYKEGYGEGCVTIHEIENNTDELKFSNCVEEEVYPNNTVTCNDYTATQEEYEGTYTSRNRGYDGAYESNSSVPADYASAYEEKAYTDGRRDNPCESNRGYGDYTPLPAGYVTKELEYFPETDKVWIEIGETEGTFIVDSVELLLMEE

SEQ ID NO: 5 - DNA, 1812 bp, artificial
  Cry1Da2 v4 DNA from pDAB109841 (truncated Cry1Da; maize optimized)
atggagatcaacaaccagaatcagtgcgttccttacaactgtctgagcaaccccaaagaaatcatccttggcgaggagaggctggaaactggcaacacagtggctgacattagcttgggtcttatcaacttcttgtactcaaactttgttcccggtggaggcttcattgtgggactgcttgagctgatatggggtttcataggtccgagccagtgggacatctttctggcacaaatcgagcagctcatctcacagcggattgaggagtttgcgagaaatcaagccatatcgagactcgaagggctgtccaacttgtacaaggtctatgtgagggctttctctgattgggagaaggaccccacgaatccagcgcttcgcgaggagatgaggatacagttcaatgacatgaactctgcgttgatcacggctattccgctctttagggtgcagaactacgaggttgctctgctctcagtgtacgtgcaagctgccaacttgcatctgagcatcctccgggacgtctcggtgtttggggaacggtggggttatgacaccgcaacgatcaacaaccgctattcagaccttacatctcttatccacgtgtacacgaatcactgcgttgatacgtacaatcaaggcctccgcagactcgaagggaggttcctcagcgattggattgtttacaatcgcttcagacggcaactcacaatctcggttctggacatagtcgcgttcttcccgaactatgatatccgcacctatcccattcagaccgctactcagctcactcgcgaagtgtatcttgacctcccgttcatcaatgagaacttgtcaccagcagcgtcctatcccaccttctcagctgcggagtccgctatcatccgctccccacatctggttgatttcctcaactctttcactatctacaccgactcgcttgcgagatacgcatactggggtggccatctggtgaactcattccggactggcaccacgaccaatctgatccgcagccctctctacggacgcgagggcaacaccgagaggccagtgaccatcaccgcttccccttccgttcctatcttccgcaccctttcgtacattactggcctcgacaacagcaacccagtcgctggcatcgagggtgttgagtttcagaacaccatttctaggtctatctataggaagagcggtccaatagactcgttttctgagttgcctccccaagatgcctctgtcagcccagccattggctactcccatcggctctgtcacgccaccttccttgaacgcatctccggaccaaggatcgctgggacggtctttagctggacccaccgctcagcatctccgacaaatgaggtctccccttcccgcatcacacaaatcccgtgggtgaaggcacacacattggcctcgggagcctcggtcatcaaagggcctggcttcactggaggcgacattctgacgaggaactcaatgggtgagctggggaccttgagggtcactttcactggacgcctcccacagtcctactacattcggttccgctatgccagcgtggccaataggtccggaacattccgctacagccagccacccagctacggcattagcttccctaagactatggatgctggggaacctctgacctcaaggtcgtttgcccacacgacgctgttcacccctatcacattcagcagagcacaagaggagtttgatctgtacatccagtccggagtctacattgaccggatcgagttcattccggttactgcgacactcgaggctgaatcggatcttgaaaggtga

SEQ ID NO: 6 - protein, 603 aa, artificial
  Cry1Da2 v4 protein (truncated Cry1Da)
MEINNQNQCVPYNCLSNPKEIILGEERLETGNTVADISLGLINFLYSNFVPGGGFIVGLLELIWGFIGPSQWDIFLAQIEQLISQRIEEFARNQAISRLEGLSNLYKVYVRAFSDWEKDPTNPALREEMRIQFNDMNSALITAIPLFRVQNYEVALLSVYVQAANLHLSILRDVSVFGERWGYDTATINNRYSDLTSLIHVYTNHCVDTYNQGLRRLEGRFLSDWIVYNRFRRQLTISVLDIVAFFPNYDIRTYPIQTATQLTREVYLDLPFINENLSPAASYPTFSAAESAIIRSPHLVDFLNSFTIYTDSLARYAYWGGHLVNSFRTGTTTNLIRSPLYGREGNTERPVTITASPSVPIFRTLSYITGLDNSNPVAGIEGVEFQNTISRSIYRKSGPIDSFSELPPQDASVSPAIGYSHRLCHATFLERISGPRIAGTVFSWTHRSASPTNEVSPSRITQIPWVKAHTLASGASVIKGPGFTGGDILTRNSMGELGTLRVTFTGRLPQSYYIRFRYASVANRSGTFRYSQPPSYGISFPKTMDAGEPLTSRSFAHTTLFTPITFSRAQEEFDLYIQSGVYIDRIEFIPVTATLEAESDLER

SEQ ID NO: 7 - DNA, 20 bp, artificial
  AAD1F Primer
tgttcggttccctctaccaa

SEQ ID NO: 8 - DNA, 22 bp, artificial
  AAD1R Primer
caacatccatcaccttgactga

SEQ ID NO: 9 - DNA, 24 bp, artificial
  AAD1P Probe
cacagaaccgtcgcttcagcaaca

SEQ ID NO: 10 - DNA, 19 bp, artificial
  SPC1A Primer
cttagctggataacgccac

SEQ ID NO: 11 - DNA, 19 bp, artificial
  SPC1S Primer
gaccgtaaggcttgatgaa

SEQ ID NO: 12 - DNA, 21 bp, artificial
  TQSPC Probe
cgagattctccgcgctgtaga

SEQ ID NO: 13 - DNA, 18 bp, artificial
  InvertaseF Primer
tggcggacgacgacttgt

SEQ ID NO: 14 - DNA, 19 bp, artificial
  InvertaseR Primer
aaagtttggaggctgccgt

SEQ ID NO: 15 - DNA, 21 bp, artificial
  InvertaseP Probe
cgagcagaccgccgtgtactt